European Patent Specification EP 4 499 875 B1, published March 12, 2025. Title: BIOMARKERS OF IL7R MODULATOR ACTIVITY. Applicant: OSE IMMUNOTHERAPEUTICS. Application WO. The sequence listing filed with the application follows.

SEQUENCE LISTING (26 sequences)

SEQ ID NO: 1 - protein, 9 aa, synthetic construct
  REGION 1..9: note = VHCDR1
FTLSDYYMA

SEQ ID NO: 2 - protein, 17 aa, synthetic construct
  REGION 1..17: note = VH CDR2
TISASGLRTYYPDSVKG

SEQ ID NO: 3 - protein, 13 aa, synthetic construct
  REGION 1..13: note = VH CDR3
PLSAHYGFNYFDY

SEQ ID NO: 4 - protein, 12 aa, synthetic construct
  REGION 1..12: note = VL CDR1
CRTSEDIYQGLA

SEQ ID NO: 5 - protein, 7 aa, synthetic construct
  REGION 1..7: note = VL CDR2
SANTLHI

SEQ ID NO: 6 - protein, 9 aa, synthetic construct
  REGION 1..9: note = VL CDR3
QQYYDYPLA

SEQ ID NO: 7 - protein, 122 aa, synthetic construct
  REGION 1..122: note = N13B2-hVL6 VH
QVQLVESGGGLVKPGGSLRLSCAVSGFTLSDYYMAWIRQAPGKGLEWVSTISASGLRTYYPDSVKGRFTISRDNAKNSLYLQMNSLRAEDTAVYYCARPLSAHYGFNYFDYWGQGTLVTVSS

SEQ ID NO: 8 - protein, 107 aa, synthetic construct
  REGION 1..107: note = N13B2-hVL6 VL
DIQMTQSPSSLSASVGDRVTITCRTSEDIYQGLAWYQQKPGKAPKLLLYSANTLHIGVPSRFSGSGSGTDYTLTISSLQPEDFATYYCQQYYDYPLAFGGGTKVEIK

SEQ ID NO: 9 - protein, 449 aa, synthetic construct
  REGION 1..449: note = N13B2-hVL6 full heavy chain
QVQLVESGGGLVKPGGSLRLSCAVSGFTLSDYYMAWIRQAPGKGLEWVSTISASGLRTYYPDSVKGRFTISRDNAKNSLYLQMNSLRAEDTAVYYCARPLSAHYGFNYFDYWGQGTLVTVSSASTKGPSVFPLAPCSRSTSESTAALGCLVKDYFPEPVTVSWNSGALTSGVHTFPAVLQSSGLYSLSSVVTVPSSSLGTKTYTCNVDHKPSNTKVDKRVESKYGPPCPPCPAPEFLGGPSVFLFPPKPKDTLMISRTPEVTCVVVDVSQEDPEVQFNWYVDGVEVHNAKTKPREEQFNSTYRVVSVLTVLHQDWLNGKEYKCKVSNKGLPSSIEKTISKAKGQPREPQVYTLPPSQEEMTKNQVSLTCLVKGFYPSDIAVEWESNGQPENNYKTTPPVLDSDGSFFLYSRLTVDKSRWQEGNVFSCSVMHEALHNHYTQKSLSLSPGK

SEQ ID NO: 10 - protein, 214 aa, synthetic construct
  REGION 1..214: note = N13B2-hVL6 full light chain
DIQMTQSPSSLSASVGDRVTITCRTSEDIYQGLAWYQQKPGKAPKLLLYSANTLHIGVPSRFSGSGSGTDYTLTISSLQPEDFATYYCQQYYDYPLAFGGGTKVEIKRTVAAPSVFIFPPSDEQLKSGTASVVCLLNNFYPREAKVQWKVDNALQSGNSQESVTEQDSKDSTYSLSSTLTLSKADYEKHKVYACEVTHQGLSSPVTKSFNRGEC

SEQ ID NO: 11 - protein, 13 aa, synthetic construct
  REGION 1..13: note = MD3 HDCR3a
PMSAHYGFNYFDY

SEQ ID NO: 12 - protein, 11 aa, synthetic construct
  REGION 1..11: note = MD3 HLCDR1a
RTSEDIYNGLA

SEQ ID NO: 13 - protein, 7 aa, synthetic construct
  REGION 1..7: note = MD3 HLCDR2a
SANSLHI

SEQ ID NO: 14 - protein, 122 aa, synthetic construct
  REGION 1..122: note = MD3 VH N13B2
AVQLVESGGGLVQPGGSLKLSCAVSGFTLSDYYMAWVRQAPKKGLEWVATISASGLRTYYPDSVKGRFTISRDDAKRSLFLQMTSLKSEDTATYYCARPMSAHYGFNYFDYWGQGVMVTVSS

SEQ ID NO: 15 - protein, 122 aa, synthetic construct
  REGION 1..122: note = MD3 VH N13B2h1
QVQLVESGGGLVKPGGSLRLSCAVSGFTLSDYYMAWVRQAPGKGLEWVATISASGLRTYYPDSVKGRFTISRDDAKNSLYLQMNSLRAEDTAVYYCARPMSAHYGFNYFDYWGQGTLVTVSS

SEQ ID NO: 16 - protein, 122 aa, synthetic construct
  REGION 1..122: note = MD3 VH N13B2h2
QVQLVESGGGLVKPGGSLRLSCAVSGFTLSDYYMAWIRQAPGKGLEWVSTISASGLRTYYPDSVKGRFTISRDNAKNSLYLQMNSLRAEDTAVYYCARPMSAHYGFNYFDYWGQGTLVTVSS

SEQ ID NO: 17 - protein, 122 aa, synthetic construct; identical to SEQ ID NO: 7
  REGION 1..122: note = MD3 VH N13B2h3

SEQ ID NO: 18 - protein, 108 aa, synthetic construct
  REGION 1..108: note = MD3 VL N13B2
DIQMTQSPASLSASLGETVTIECRTSEDIYNGLAWYQQKPGKSPQLLVYSANSLHIGVPSRFSGSGSGTQYSLKINSLQFEDVASYFCQQYYDYPLAFGSGTKLEIKR

SEQ ID NO: 19 - protein, 107 aa, synthetic construct
  REGION 1..107: note = MD3 VL N13B2h1
EIVMTQSPATLSVSPGERATLSCRTSEDIYNGLAWYQQKPGQAPRLLVYSANSLHIGIPARFSGSGSGTEYTLTISSLQSEDFAVYFCQQYYDYPLAFGGGTKVEIK

SEQ ID NO: 20 - protein, 107 aa, synthetic construct
  REGION 1..107: note = MD3 VL N13B2h2
EIVMTQSPATLSVSPGERATLSCRTSEDIYNGLAWYQQKPGQAPRLLIYSANSLHIGIPARFSGSGSGTEFTLTISSLQSEDFAVYYCQQYYDYPLAFGGGTKVEIK

SEQ ID NO: 21 - protein, 107 aa, synthetic construct
  REGION 1..107: note = MD3 VL N13B2h3
EIVMTQSPATLSVSPGERATLSCRTSEDIYQGLAWYQQKPGQAPRLLIYSANTLHIGIPARFSGSGSGTEFTLTISSLQSEDFAVYYCQQYYDYPLAFGGGTKVEIK

SEQ ID NO: 22 - protein, 449 aa, synthetic construct; identical to SEQ ID NO: 9
  REGION 1..449: note = MD3 N13B2h3 Full heavy chain

SEQ ID NO: 23 - protein, 213 aa, synthetic construct
  REGION 1..213: note = MD3 N13B2h3 Full light chain
EIVMTQSPATLSVSPGERATLSCRTSEDIYQGLAWYQQKPGQAPRLLIYSANTLHIGIPARFSGSGSGTEFTLTISSLQSEDFAVYYCQQYYDYPLAFGGGTKVEIKTVAAPSVFIFPPSDEQLKSGTASVVCLLNNFYPREAKVQWKVDNALQSGNSQESVTEQDSKDSTYSLSSTLTLSKADYEKHKVYACEVTHQGLSSPVTKSFNRGEC

SEQ ID NO: 24 - protein, 107 aa, synthetic construct
  REGION 1..107: note = MD5 VL1
DIQMTQSPSSLSASVGDRVTITCRTSEDIYQGLAWYQQKPGKAPKLLVYSANTLHIGVPSRFSGSGSGTDYTLTISSLQPEDFATYFCQQYYDYPLAFGGGTKVEIK

SEQ ID NO: 25 - protein, 107 aa, synthetic construct
  REGION 1..107: note = MD5 VL2
DIQMTQSPSSLSASVGDRVTITCRTSEDIYQGLAWYQQKPGKAPKLLLYSANTLHIGVPSRFSGSGSGTDYTLTISSLQPEDFATYFCQQYYDYPLAFGGGTKVEIK

SEQ ID NO: 26 - protein, 107 aa, synthetic construct
  REGION 1..107: note = MD5 VL3
DIQMTQSPSSLSASVGDRVTITCRTSEDIYQGLAWYQQKPGKAPKLLVYSANTLHIGVPSRFSGSGSGTDYTLTISSLQPEDFATYYCQQYYDYPLAFGGGTKVEIK